European Patent Specification EP 3 542 808 B1, published March 19, 2025. Title: THERAPEUTIC VIRAL MICROPARTICLES FOR PROMOTING STENT BIOFUNCTIONALITY AND WOUND HEALING IN VERTEBRATE INDIVIDUALS. Applicant: MANGOGEN PHARMA INC. The sequence listing filed with the application follows.

SEQUENCE LISTING (2 sequences)

SEQ ID NO: 1 - DNA, 22 bp, Artificial Sequence
  Oligonucleotide
cttgccttgctgctctacctcc

SEQ ID NO: 2 - DNA, 22 bp, Artificial Sequence
  Oligonucleotide
gctgcgctgatagacatccatg